European Patent Specification EP 3 717 020 B1, published February 21, 2024. Title: RAS-TARGETED THERAPEUTIC. Applicant: The Hospital For Sick Children. Application To be assigned. The sequence listing filed with the application follows.

SEQUENCE LISTING (30 sequences)

SEQ ID NO: 1 - protein, 199 aa, Corynebacterium diphtheriae
  MISC_FEATURE: dtA Domain
GADDVVDSSKSFVMENFSSYHGTKPGYVDSIQKGIQKPKSGTQGNYDDDWKGFYSTDNKYDAAGYSVDNENPLSGKAGGVVKVTYPGLTKVLALKVDNAETIKKELGLSLTEPLMEQVGTEEFIKRFGDGASRVVLSLPFAEGSSSVEYINNWEQAKALSVELEINFETRGKRGQDAMYEYMAQACAGNRVRRSVGSSL

SEQ ID NO: 2 - protein, 199 aa, Corynebacterium diphtheriae
  MISC_FEATURE: dta Domain (K51E, E148K)
GADDVVDSSKSFVMENFSSYHGTKPGYVDSIQKGIQKPKSGTQGNYDDDWEGFYSTDNKYDAAGYSVDNENPLSGKAGGVVKVTYPGLTKVLALKVDNAETIKKELGLSLTEPLMEQVGTEEFIKRFGDGASRVVLSLPFAEGSSSVKYINNWEQAKALSVELEINFETRGKRGQDAMYEYMAQACAGNRVRRSVGSSL

SEQ ID NO: 3 - protein, 339 aa, Corynebacterium diphtheriae
  MISC_FEATURE: dtB Domain
SCINLDWDVIRDKTKTKIESLKEHGPIKNKMSESPNKTVSEEKAKQYLEEFHQTALEHPELSELKTVTGTNPVFAGANYAAWAVNVAQVIDSETADNLEKTTAALSILPGIGSVMGIADGAVHHNTEEIVAQSIALSSLMVAQAIPLVGELVDIGFAAYNFVESIINLFQVVHNSYNRPAYSPGHKTQPFLHDGYAVSWNTVEDSIIRTGFQGESGHDIKITAENTPLPIAGVLLPTIPGKLDVNKSKTHISVNGRKIRMRCRAIDGDVTFCRPKSPVYVGNGVHANLHVAFHRSSSEKIHSNEISSDSIGVLGYQKTVDHTKVNSKLSLFFEIKSRQA

SEQ ID NO: 4 - protein, 179 aa, Corynebacterium diphtheriae
  MISC_FEATURE: dtT (dtB Translocation Domain)
SCINLDWDVIRDKTKTKIESLKEHGPIKNKMSESPNKTVSEEKAKQYLEEFHQTALEHPELSELKTVTGTNPVFAGANYAAWAVNVAQVIDSETADNLEKTTAALSILPGIGSVMGIADGAVHHNTEEIVAQSIALSSLMVAQAIPLVGELVDIGFAAYNFVESIINLFQVVHNSYNRP

SEQ ID NO: 5 - protein, 179 aa, Corynebacterium diphtheriae
  MISC_FEATURE: Translocation-deficient dtT (L350K)
SCINLDWDVIRDKTKTKIESLKEHGPIKNKMSESPNKTVSEEKAKQYLEEFHQTALEHPELSELKTVTGTNPVFAGANYAAWAVNVAQVIDSETADNLEKTTAALSILPGIGSVMGIADGAVHHNTEEIVAQSIALSSLMVAQAIPLVGEKVDIGFAAYNFVESIINLFQVVHNSYNRP

SEQ ID NO: 6 - protein, 160 aa, Corynebacterium diphtheriae
  MISC_FEATURE: dtR (dtB Receptor-binding Domain)
AYSPGHKTQPFLHDGYAVSWNTVEDSIIRTGFQGESGHDIKITAENTPLPIAGVLLPTIPGKLDVNKSKTHISVNGRKIRMRCRAIDGDVTFCRPKSPVYVGNGVHANLHVAFHRSSSEKIHSNEISSDSIGVLGYQKTVDHTKVNSKLSLFFEIKSRQA

SEQ ID NO: 7 - protein, 119 aa, Artificial Sequence
  Polyhistidine-SUMO
MGSSHHHHHHGSGLVPRGSASMSDSEVNQEAKPEVKPEVKPETHINLKVSDGSSEIFFKIKKTTPLRRLMEAFAKRQGKEMDSLRFLYDGIRIQADQTPEDLDMEDNDIIEAHREQIGG

SEQ ID NO: 8 - protein, 10 aa, Artificial Sequence
  MYC tag
EQKLISEEDL

SEQ ID NO: 9 - protein, 9 aa, Artificial Sequence
  SV40 nuclear localization sequences (NLS)
SPPKKKRKV

SEQ ID NO: 10 - protein, 5 aa, Artificial Sequence
  (G4S) linker
GGGGS

SEQ ID NO: 11 - protein, 10 aa, Artificial Sequence
  (G4S)2 linker
GGGGSGGGGS

SEQ ID NO: 12 - protein, 15 aa, Artificial Sequence
  (G4S)3 linker
GGGGSGGGGSGGGGS

SEQ ID NO: 13 - protein, 238 aa, Aequorea victoria
  MISC_FEATURE: Enhanced Green Fluorescent Protein (eGFP)
GSKGEELFTGVVPILVELDGDVNGHKFSVSGEGEGDATYGKLTLKFICTTGKLPVPWPTLVTTLTYGVQCFSRYPDHMKQHDFFKSAMPEGYVQERTIFFKDDGNYKTRAEVKFEGDTLVNRIELKGIDFKEDGNILGHKLEYNYNSHNVYIMADKQKNGIKVNFKIRHNIEDGSVQLADHYQQNTPIGDGPVLLPDNHYLSTQSALSKDPNEKRDHMVLLEFVTAAGITLGMDELYK

SEQ ID NO: 14 - protein, 235 aa, Discosoma sp. (also: Actinodiscus or mushroom coral)
  MISC_FEATURE: Monomeric Cherry (mCherry)
GSKGEEDNMAIIKEFMRFKVHMEGSVNGHEFEIEGEGEGRPYEGTQTAKLKVTKGGPLPFAWDILSPQFMYGSKAYVKHPADIPDYLKLSFPEGFKWERVMNFEDGGVVTVTQDSSLQDGEFIYKVKLRGTNFPSDGPVMQKKTMGWEASSERMYPEDGALKGEIKQRLKLKDGGHYDAEVKTTYKAKKPVQLPGAYNVNIKLDITSHNEDYTIVEQYERAEGRHSTGGMDELYK

SEQ ID NO: 15 - protein, 493 aa, Bacillus megaterium
  MISC_FEATURE: alpha-amylase (B. megaterium)
GHKGKSPTADKNGVFYEVYVNSFYDANKDGHGDLKGLTQKLDYLNDGNSHTKNDLQVNGIWMMPVNPSPSYHKYDVTDYYNIDPQYGNLQDFRKLMKEADKRDVKVIMDLVVNHTSSEHPWFQAALKDKNSKYRDYYIWADKNTDLNEKGSWGQQVWHKAPNGEYFYGTFWEGMPDLNYDNPEVRKEMINVGKFWLNQGVDGFRLDAALHIFKGQTPEGAKKNILWWNEFRDAMKKENPNVYLTGEVWDQPEVVAPYYQSLDSLFNFDLAGKIVSSVKAGNDQGIATAAAATDELFKSYNPNKIDGIFLTNHDQNRVMSELSGDVNKAKSAASILLTLPGNPYIYYGEEIGMTGEKPDELIREPFRWYEGNGLGQTSWETPIYNKGGNGVSIEAQTKQKDSLLNHYREMIRVRQQHEELVKGTLQSISLDQKEVVAYSRTYKGKSISVYHNISNQPIKVSVAAKGKLIFSSEKGVKKVKNQLVIPANTTILIK

SEQ ID NO: 16 - protein, 497 aa, Homo sapiens
  MISC_FEATURE: MeCP2 (e1 isoform)
AAAAAAAPSGGGGGGEEERLEEKSEDQDLQGLKDKPLKFKKVKKDKKEEKEGKHEPVQPSAHHSAEPAEAGKAETSEGSGSAPAVPEASASPKQRRSIIRDRGPMYDDPTLPEGWTRKLKQRKSGRSAGKYDVYLINPQGKAFRSKVELIAYFEKVGDTSLDPNDFDFTVTGRGSPSRREQKPPKKPKSPKAPGTGRGRGRPKGSGTTRPKAATSEGVQVKRVLEKSPGKLLVKMPFQTSPGGKAEGGGATTSTQVMVIKRPGRKRKAEADPQAIPKKRGRKPGSVVAAAAAEAKKKAVKESSIRSVQETVLPIKKRKTRETVSIEVKEVVKPLLVSTLGEKSGKGLKTCKSPGRKSKESSPKGRSSSASSPPKKEHHHHHHHSESPKAPVPLLPPLPPPPPEPESSEDPTSPPEPQDLSSSVCKEEKMPRGGSLESDGCPKEPAKTQPAVATAATAAEKYKHRGEGERKDIVSSSMPRPNREEPVDSRTPVTERVS

SEQ ID NO: 17 - protein, 485 aa, Homo sapiens
  MISC_FEATURE: MeCP2 (e2 isoform)
VAGMLGLREEKSEDQDLQGLKDKPLKFKKVKKDKKEEKEGKHEPVQPSAHHSAEPAEAGKAETSEGSGSAPAVPEASASPKQRRSIIRDRGPMYDDPTLPEGWTRKLKQRKSGRSAGKYDVYLINPQGKAFRSKVELIAYFEKVGDTSLDPNDFDFTVTGRGSPSRREQKPPKKPKSPKAPGTGRGRGRPKGSGTTRPKAATSEGVQVKRVLEKSPGKLLVKMPFQTSPGGKAEGGGATTSTQVMVIKRPGRKRKAEADPQAIPKKRGRKPGSVVAAAAAEAKKKAVKESSIRSVQETVLPIKKRKTRETVSIEVKEVVKPLLVSTLGEKSGKGLKTCKSPGRKSKESSPKGRSSSASSPPKKEHHHHHHHSESPKAPVPLLPPLPPPPPEPESSEDPTSPPEPQDLSSSVCKEEKMPRGGSLESDGCPKEPAKTQPAVATAATAAEKYKHRGEGERKDIVSSSMPRPNREEPVDSRTPVTERVS

SEQ ID NO: 18 - protein, 585 aa, Homo sapiens
  MISC_FEATURE: FMRP
EELVVEVRGSNGAFYKAFVKDVHEDSITVAFENNWQPDRQIPFHDVRFPPPVGYNKDINESDEVEVYSRANEKEPCCWWLAKVRMIKGEFYVIEYAACDATYNEIVTIERLRSVNPNKPATKDTFHKIKLDVPEDLRQMCAKEAAHKDFKKAVGAFSVTYDPENYQLVILSINEVTSKRAHMLIDMHFRSLRTKLSLIMRNEEASKQLESSRQLASRFHEQFIVREDLMGLAIGTHGANIQQARKVPGVTAIDLDEDTCTFHIYGEDQDAVKKARSFLEFAEDVIQVPRNLVGKVIGKNGKLIQEIVDKSGVVRVRIEAENEKNVPQEEEIMPPNSLPSNNSRVGPNAPEEKKHLDIKENSTHFSQPNSTKVQRGMVPFVFVGTKDSIANATVLLDYHLNYLKEVDQLRLERLQIDEQLRQIGASSRPPPNRTDKEKSYVTDDGQGMGRGSRPYRNRGHGRRGPGYTSAPTEEERESFLRRGDGRRRGGGGRGQGGRGRGGGFKGNDDHSRTDNRPRNPREAKGRTTDGSLQIRVDCNNERSVHTKTLQNTSSEGSRLRTGKDRNQKKEKPDSVDGQQPLVNGVP

SEQ ID NO: 19 - protein, 294 aa, Homo sapiens
  MISC_FEATURE: SMN protein
MAMSSGGSGGGVPEQEDSVLFRRGTGQSDDSDIWDDTALIKAYDKAVASFKHALKNGDICETSGKPKTTPKRKPAKKNKSQKKNTAASLQQWKVGDKCSAIWSEDGCIYPATIASIDFKRETCVVVYTGYGNREEQNLSDLLSPICEVANNIEQNAQENENESQVSTDESENSRSPGNKSDNIKPKSAPWNSFLPPPPPMPGPRLGPGKPGLKFNGPPPPPPPPPPHLLSCWLPPFPSGPPIIPPPPPICPDSLDDADALGSMLISWYMSGYHTGYYMGFRQNQKEGRCSHSLN

SEQ ID NO: 20 - protein, 261 aa, Clostridium difficile
  MISC_FEATURE: CPD (C. difficile)
EGSLGEDDNLDFSQNIVVDKEYLLEKISSLARSSERGYIHYIVQLQGDKISYEAACNLFAKTPYDSVLFQKNIEDSEIAYYYNPGDGEIQEIDKYKIPSIISDRPKIKLTFIGHGKDEFNTDIFAGFDVDSLSTEIEAAIDLAKEDISPKSIEINLLGCNMFSYSINVEETYPGKLLLKVKDKISELMPSISQDSIIVSANQYEVRINSEGRRELLDHSGEWINKEESIIKDISSKEYISFNPKENKITVKSKNLPELSTL

SEQ ID NO: 21 - protein, 212 aa, Vibrio cholerae
  MISC_FEATURE: CPD (V. cholera)
KEALADGKILHNQNVNSWGPITVTPTTDGGETRFDGQIIVQMENDPVVAKAAANLAGKHAESSVVVQLDSDGNYRVVYGDPSKLDGKLRWQLVGHGRDHSETNNTRLSGYSADELAVKLAKFQQSFNQAENINNKPDHISIVGCSLVSDDKQKGFGHQFINAMDANGLRVDVSVRSSELAVDEAGRKHTKDANGDWVQKAENNKVSLSWDAQ

SEQ ID NO: 22 - protein, 1371 aa, Streptococcus pyogenes
  MISC_FEATURE: Cas9 (S. pyogenes)
MDKKYSIGLDIGTNSVGWAVITDDYKVPSKKFKVLGNTDRHSIKKNLIGALLFGSGETAEATRLKRTARRRYTRRKNRICYLQEIFSNEMAKVDDSFFHRLEESFLVEEDKKHERHPIFGNIVDEVAYHEKYPTIYHLRKKLADSTDKADLRLIYLALAHMIKFRGHFLIEGDLNPDNSDVDKLFIQLVQIYNQLFEENPINASRVDAKAILSARLSKSRRLENLIAQLPGEKRNGLFGNLIALSLGLTPNFKSNFDLAEDAKLQLSKDTYDDDLDNLLAQIGDQYADLFLAAKNLSDAILLSDILRVNSEITKAPLSASMIKRYDEHHQDLTLLKALVRQQLPEKYKEIFFDQSKNGYAGYIDGGASQEEFYKFIKPILEKMDGTEELLVKLNREDLLRKQRTFDNGSIPHQIHLGELHAILRRQEDFYPFLKDNREKIEKILTFRIPYYVGPLARGNSRFAWMTRKSEETITPWNFEEVVDKGASAQSFIERMTNFDKNLPNEKVLPKHSLLYEYFTVYNELTKVKYVTEGMRKPAFLSGEQKKAIVDLLFKTNRKVTVKQLKEDYFKKIECFDSVEISGVEDRFNASLGAYHDLLKIIKDKDFLDNEENEDILEDIVLTLTLFEDRGMIEERLKTYAHLFDDKVMKQLKRRRYTGWGRLSRKLINGIRDKQSGKTILDFLKSDGFANRNFMQLIHDDSLTFKEDIQKAQVSGQGHSLHEQIANLAGSPAIKKGILQTVKIVDELVKVMGHKPENIVIEMARENQTTQKGQKNSRERMKRIEEGIKELGSQILKEHPVENTQLQNEKLYLYYLQNGRDMYVDQELDINRLSDYDVDHIVPQSFIKDDSIDNKVLTRSDKNRGKSDNVPSEEVVKKMKNYWRQLLNAKLITQRKFDNLTKAERGGLSELDKAGFIKRQLVETRQITKHVAQILDSRMNTKYDENDKLIREVKVITLKSKLVSDFRKDFQFYKVREINNYHHAHDAYLNAVVGTALIKKYPKLESEFVYGDYKVYDVRKMIAKSEQEIGKATAKYFFYSNIMNFFKTEITLANGEIRKRPLIETNGETGEIVWDKGRDFATVRKVLSMPQVNIVKKTEVQTGGFSKESILPKRNSDKLIARKKDWDPKKYGGFDSPTVAYSVLVVAKVEKGKSKKLKSVKELLGITIMERSSFEKNPIDFLEAKGYKEVKKDLIIKLPKYSLFELENGRKRMLASAGELQKGNELALPSKYVNFLYLASHYEKLKGSPEDNEQKQLFVEQHKHYLDEIIEQISEFSKRVILADANLDKVLSAYNKHRDKPIREQAENIIHLFTLTNLGAPAAFKYFDTTIDRKRYTSTKEVLDATLIHQSITGLYETRIDLSQLGGDSPVR

SEQ ID NO: 23 - protein, 1403 aa, Artificial Sequence
  Cas9 (S. pyogenes) with N-terminal His, SV40 and C-terminal SV40 sequences
HHHHHHGSGATMASPPKKKRKVGSMDKKYSIGLDIGTNSVGWAVITDDYKVPSKKFKVLGNTDRHSIKKNLIGALLFGSGETAEATRLKRTARRRYTRRKNRICYLQEIFSNEMAKVDDSFFHRLEESFLVEEDKKHERHPIFGNIVDEVAYHEKYPTIYHLRKKLADSTDKADLRLIYLALAHMIKFRGHFLIEGDLNPDNSDVDKLFIQLVQIYNQLFEENPINASRVDAKAILSARLSKSRRLENLIAQLPGEKRNGLFGNLIALSLGLTPNFKSNFDLAEDAKLQLSKDTYDDDLDNLLAQIGDQYADLFLAAKNLSDAILLSDILRVNSEITKAPLSASMIKRYDEHHQDLTLLKALVRQQLPEKYKEIFFDQSKNGYAGYIDGGASQEEFYKFIKPILEKMDGTEELLVKLNREDLLRKQRTFDNGSIPHQIHLGELHAILRRQEDFYPFLKDNREKIEKILTFRIPYYVGPLARGNSRFAWMTRKSEETITPWNFEEVVDKGASAQSFIERMTNFDKNLPNEKVLPKHSLLYEYFTVYNELTKVKYVTEGMRKPAFLSGEQKKAIVDLLFKTNRKVTVKQLKEDYFKKIECFDSVEISGVEDRFNASLGAYHDLLKIIKDKDFLDNEENEDILEDIVLTLTLFEDRGMIEERLKTYAHLFDDKVMKQLKRRRYTGWGRLSRKLINGIRDKQSGKTILDFLKSDGFANRNFMQLIHDDSLTFKEDIQKAQVSGQGHSLHEQIANLAGSPAIKKGILQTVKIVDELVKVMGHKPENIVIEMARENQTTQKGQKNSRERMKRIEEGIKELGSQILKEHPVENTQLQNEKLYLYYLQNGRDMYVDQELDINRLSDYDVDHIVPQSFIKDDSIDNKVLTRSDKNRGKSDNVPSEEVVKKMKNYWRQLLNAKLITQRKFDNLTKAERGGLSELDKAGFIKRQLVETRQITKHVAQILDSRMNTKYDENDKLIREVKVITLKSKLVSDFRKDFQFYKVREINNYHHAHDAYLNAVVGTALIKKYPKLESEFVYGDYKVYDVRKMIAKSEQEIGKATAKYFFYSNIMNFFKTEITLANGEIRKRPLIETNGETGEIVWDKGRDFATVRKVLSMPQVNIVKKTEVQTGGFSKESILPKRNSDKLIARKKDWDPKKYGGFDSPTVAYSVLVVAKVEKGKSKKLKSVKELLGITIMERSSFEKNPIDFLEAKGYKEVKKDLIIKLPKYSLFELENGRKRMLASAGELQKGNELALPSKYVNFLYLASHYEKLKGSPEDNEQKQLFVEQHKHYLDEIIEQISEFSKRVILADANLDKVLSAYNKHRDKPIREQAENIIHLFTLTNLGAPAAFKYFDTTIDRKRYTSTKEVLDATLIHQSITGLYETRIDLSQLGGDSPVRSPKKKRKV

SEQ ID NO: 24 - protein, 289 aa, Homo sapiens
  MISC_FEATURE: PNP
MENGYTYEDYKNTAEWLLSHTKHRPQVAIICGSGLGGLTDKLTQAQIFDYSEIPNFPRSTVPGHAGRLVFGFLNGRACVMMQGRFHMYEGYPLWKVTFPVRVFHLLGVDTLVVTNAAGGLNPKFEVGDIMLIRDHINLPGFSGQNPLRGPNDERFGDRFPAMSDAYDRTMRQRALSTWKQMGEQRELQEGTYVMVAGPSFETVAECRVLQKLGADAVGMSTVPEVIVARHCGLRVFGFSLITNKVIMDYESLEKANHEEVLAAGKQAAQKLEQFVSILMASIPLPDKAS

SEQ ID NO: 25 - protein, 98 aa, Artificial Sequence
  SUMO
MSDSEVNQEAKPEVKPEVKPETHINLKVSDGSSEIFFKIKKTTPLRRLMEAFAKRQGKEMDSLRFLYDGIRIQADQTPEDLDMEDNDIIEAHREQIGG

SEQ ID NO: 26 - protein, 14 aa, Corynebacterium diphtheriae
  MISC_FEATURE: delta-dta
CAGNRVRRSVGSSL

SEQ ID NO: 27 - protein, 15 aa, Artificial Sequence
  Strep Tag (TM) II
LVPRGSAWSHPQFEK

SEQ ID NO: 28 - protein, 543 aa, Clostridium difficile
  MISC_FEATURE: contains glucosyl transferase domain
MSLVNRKQLEKMANVRFRTQEDEYVAILDALEEYHNMSENTVVEKYLKLKDINSLTDIYIDTYKKSGRNKALKKFKEYLVTEVLELKNNNLTPVEKNLHFVWIGGQINDTAINYINQWKDVNSDYNVNVFYDSNAFLINTLKKTVVESAINDTLESFRENLNDPRFDYNKFFRKRMEIIYDKQKNFINYYKAQREENPELIIDDIVKTYLSNEYSKEIDELNTYIEESLNKITQNSGNDVRNFEEFKNGESFNLYEQELVERWNLAAASDILRISALKEIGGMYLDVDMLPGIQPDLFESIEKPSSVTVDFWEMTKLEAIMKYKEYIPEYTSEHFDMLDEEVQSSFESVLASKSDKSEIFSSLGDMEASPLEVKIAFNSKGIINQGLISVKDSYCSNLIVKQIENRYKILNNSLNPAISEDNDFNTTTNTFIDSIMAEANADNGRFMMELGKYLRVGFFPDVKTTINLSGPEAYAAAYQDLLMFKEGSMNIHLIEADLRNFEISKTNISQSTEQEMASLWSFDDARAKAQFEEYKRNYFEGSL

SEQ ID NO: 29 - DNA, 1530 bp, Homo sapiens
  misc_feature: RRSP
ggtgataaaaccaaggtcgtggtcgatttagcgcaaatctttacggtgcaagagctgaaagaaagagcaaaagtttttgctaaaccgattggcgcatcctaccaaggtattctcgatcaactcgaccttgtgcatcaggctaaaggccgcgatcaaatcgcagcgagctttgagcttaataagaagattaatgactacatcgctgaacatccaacttcggggcgtaatcaagcgctaacgcagttgaaagagcaggtcaccagtgcgttgtttatcggtaagatgcaagttgcccaagcgggtattgatgcaatcgcacaaacaagaccggagcttgccgctcgtatctttatggtcgcgattgaagaagccaacggtaaacacgtaggtttgacggacatgatggttcgttgggccaatgaagacccatacttggcaccgaagcatggttacaaaggcgaaacgccaagtgaccttggttttgatgcgaagtaccacgtagatctaggtgagcattacgctgatttcaaacagtggttagaaacgtcccagtcgaacgggttgttgagtaaagcgacgttggatgaatccactaaaacggttcatcttggctatagctatcaagaacttcaggatttgacgggtgctgaatcggtgcaaatggcgttctacttcctgaaagaagcggcgaagaaagcggatccgatttctggtgattcagctgaaatgatactgctgaagaaatttgcagatcaaagctacttatctcaacttgattccgaccgaatggatcaaattgaaggtatctaccgcagtagccatgagacggatattgacgcttgggatcgtcgttactctggtacaggctatgatgagctgacgaataagcttgctagtgcaacgggcgttgacgagcagcttgcggttcttctggatgatcgtaaaggcctcttgattggtgaagtgcatggcagcgacgtcaacggcctacgctttgttaatgaacagatggatgcactgaaaaaacagggagtcacagtcattggccttgagcatttacgctcagaccttgcgcaaccgctgattgatcgctacctagctacgggtgtgatgtcgagtgaactaagcgcaatgctgaaaacaaagcatctcgatgtcactctttttgaaaacgcacgtgctaacggtatgcgcatcgtcgcgctggatgcaaacagctctgcgcgtccaaatgttcagggaacagaacatggtctgatgtaccgtgctggtgctgcgaacaacattgcggtggaagtattacaaaatctgcctgatggcgaaaagttcgttgctatctacggtaaagcgcatttgcagtctcacaaagggattgaagggttcgttcctggtatcacgcaccgtctcgatcttcctgcgcttaaagtcagtgactcgaaccagttcacagttgaacaagacgatgtaagtctacgtgttgtctacgatgatgttgctaacaaaccgaagatcacgttcaagggcagtttg

SEQ ID NO: 30 - protein, 510 aa, Homo sapiens
  MISC_FEATURE: RRSP
GDKTKVVVDLAQIFTVQELKERAKVFAKPIGASYQGILDQLDLVHQAKGRDQIAASFELNKKINDYIAEHPTSGRNQALTQLKEQVTSALFIGKMQVAQAGIDAIAQTRPELAARIFMVAIEEANGKHVGLTDMMVRWANEDPYLAPKHGYKGETPSDLGFDAKYHVDLGEHYADFKQWLETSQSNGLLSKATLDESTKTVHLGYSYQELQDLTGAESVQMAFYFLKEAAKKADPISGDSAEMILLKKFADQSYLSQLDSDRMDQIEGIYRSSHETDIDAWDRRYSGTGYDELTNKLASATGVDEQLAVLLDDRKGLLIGEVHGSDVNGLRFVNEQMDALKKQGVTVIGLEHLRSDLAQPLIDRYLATGVMSSELSAMLKTKHLDVTLFENARANGMRIVALDANSSARPNVQGTEHGLMYRAGAANNIAVEVLQNLPDGEKFVAIYGKAHLQSHKGIEGFVPGITHRLDLPALKVSDSNQFTVEQDDVSLRVVYDDVANKPKITFKGSL